European Patent Application EP 4 249 505 A1, published September 27, 2023. Title: LONG-ACTING GLUCAGON DERIVATIVE. Applicant: ZHEJIANG DOER BIOLOGICS CO., LTD. ZHEJIANG HEZE PHARMACEUTICAL TECHNOLOGY CO., LTD. The sequence listing filed with the application follows.

SEQUENCE LISTING (10 sequences)

SEQ ID NO: 1 - protein, 29 aa, Artificial Sequence
HSQGTFTSDYSKYLDSRRAQDFVQWLMNT

SEQ ID NO: 2 - protein, 31 aa, Artificial Sequence
HAEGTFTSDVSSYLEGQAAKEFIAWLVKGRG

SEQ ID NO: 3 - protein, 39 aa, Artificial Sequence
HXQGTFTSDKSKYLDSQAAQDFVQWLLAGGPSSGAPPPS

SEQ ID NO: 4 - protein, 39 aa, Artificial Sequence
HXQGTFTSDKSKXLDSQAAQDFVQWLLAGGPSSGAPPPS

SEQ ID NO: 5 - protein, 39 aa, Artificial Sequence
HXQGTFTSDYSKXKDSQAAQDFVQWLLAGGPSSGAPPPS

SEQ ID NO: 6 - protein, 39 aa, Artificial Sequence; identical to SEQ ID NO: 3

SEQ ID NO: 7 - protein, 39 aa, Artificial Sequence; identical to SEQ ID NO: 4

SEQ ID NO: 8 - protein, 39 aa, Artificial Sequence; identical to SEQ ID NO: 5

SEQ ID NO: 9 - protein, 39 aa, Artificial Sequence
HXQGTFTSDXSKXXDSQAAQDFVQWLLAGGPSSGAPPPS

SEQ ID NO: 10 - protein, 42 aa, Artificial Sequence
YAEGTFISDYSIAMDKIHQQDFVNWLLAQKGKKNDWKHNITQ